European Patent Specification EP 3 845 651 B1, published July 2, 2025. Title: Novel nuclease domain and use thereof. Applicant: HIROSHIMA UNIVERSITY. The sequence listing filed with the application follows.

SEQUENCE LISTING (122 sequences)

SEQ ID NO: 1 - protein, 585 aa, Bacillus sp. SGD-V-76
MATKRVVRTFGWIQNPGKFENLKRTVQVFDENSKVYKEVRDIKIPNLVKDKDVRTTLIAAMNRLENYYSYKELVGTGTSVRAQAPCDAIIQAAIQDQGNKKGYIDNWSSDGFVRWAHALGFLEYNSDKDSFYLTDIGLEYSRSTDDSLNEKIILIEALSSYPPAIRILTLLENGEHLTKFDLGKQLGFSGESGFTSLPQNLFLDALANAPSSPPTIKNSIRSDWEGSADKYARMISGWLVKMGLVAQGRKNFVVPTVGGSTRNEYISHAFKITKDGLDVLRRAKGASKHVRVPKRVYWEMFATNINDRVYVRTRRAYTLYLLMRSNTALNTVQLQVKLKALGFEELEETIENDVKGLINSGIFINVTNKGYHFKDTIKPFEIPEFGVTEPLVKGEMEKKKSDLRHKLKHVPHEYIELIEIAQDSKQNRLFEFKVVEFLKEVYDYNGKHLGGSRKPDGALYTNGLKTDYGIILDTKAYKDGYSLPISQADEMQRYVDENNNRNAIINPNEWWKVYPNSILDFKFLFVSGFFKGDYKKQLARVSNLTKRKGAVLSVEQLLLGGEKIKDGSLTLEDVGDKFNNDEIIF

SEQ ID NO: 2 - DNA, 1758 bp, Bacillus sp. SGD-V-76
atggcaacaaaacgagtggttcgtacatttggttggatacagaatccaggtaaattcgagaacctaaaacgaacagtccaagtattcgatgaaaactcaaaagtatataaagaggttagggatataaagattccaaatctagtgaaagataaagatgtaagaactactttaatagctgctatgaatcgattagaaaattattactcatataaagagttggttggtacaggtacttcagttagagctcaagcgccttgtgatgccattattcaagcagcgattcaagaccaaggtaataaaaaaggatacattgataattggtcttctgatggattcgttcgttgggcacatgcattggggtttcttgagtataactcagataaggactcattttacctaactgatattggattggaatattctcgttctacagatgattcactaaatgaaaaaatcatacttattgaagcattgtcatcatatccaccagcaattcgaatattgacattacttgaaaatggtgagcatttaacaaaattcgacctaggtaaacagttaggctttagtggagagagtggttttacttcattaccacaaaacttatttttagatgcgttagcaaatgcaccttcatcaccaccaacaattaagaattctattcgttctgattgggaaggttctgcggataaatatgcacggatgatttcaggctggcttgtaaagatggggcttgttgcacaaggtcgtaaaaattttgttgtaccaacggtaggtggttctactcgaaatgagtatatatctcatgcttttaaaattacaaaagatggtcttgatgtgttaaggagagcaaaaggtgccagtaaacatgtacgagtaccaaagcgtgtatactgggagatgttcgctaccaacattaacgatagagtgtatgtaagaacaagacgggcttatacactttacttgttaatgagaagtaacactgctctaaatactgttcaacttcaagtgaaattaaaagctttgggctttgaagaattggaagaaacaattgagaatgatgtaaaaggtttaattaactctggaatttttatcaatgtgacgaataaaggttatcattttaaagatacaattaaaccattcgaaattcctgaatttggcgtaacagaaccattagtaaagggggaaatggagaagaagaaatccgatttgcgtcataagttaaaacacgtaccgcatgaatatattgaactaatagaaattgcacaggattcaaagcaaaatcgtttgttcgaatttaaagtagttgagtttttgaaagaagtttatgattataatggaaagcacctaggggggagtcgaaaaccagatggcgcactatataccaatggtttaaaaacagattatggaataattttagataccaaagcttacaaagatggttatagtttaccaatctcccaggcagatgaaatgcagcgttatgtcgatgaaaataataatagaaatgctattattaatcctaacgaatggtggaaagtgtatcctaattctatcttggactttaaattcttattcgtaagtggtttttttaaaggtgactataaaaaacaattagctcgtgtaagtaatcttacaaagcgtaaaggtgctgtcctaagcgtagagcaactattattgggaggggaaaaaattaaagatggtagtttaacattagaagatgttggtgacaaattcaataatgatgaaattattttctaa

SEQ ID NO: 3 - protein, 579 aa, Clostridium botulinum
VESLRLSDITIRTFGWIQNPSDFSKLKKIVQLFDHTSSIHVDLKENRIPRLVEKDDGRDRFIEILNRIPLKIKYIDLVGTSFKPRSSGRCNGIAQAMIEGQGKSFTDNWTADGFIRWAHALGFIQYDYLEDEFSITQAGFDFSRSINDSEGENEILIEAMLSYPPAVRVLDLLSLGEHLTKFDIGKNLGFNGESGFTSLPLNIMLQTLADNDLVSEKTKIRQDWEGSSDKYSRMIAGWLSKLGLVKKGKKYFDVNIGGIIHREYISHAYKITGEGLKQLRRAKGTTSARRIEKRVCWEMFATKNLDRTYIRTRRAYILKFLEVSSSLITIEQIKTKLLEKGYDETVETIKSDIKGLINIGLNIQETTRGYSLKDSINDFMIPVTDLNQIVKSSIEMSKANMRDNLQMLPHDYIELIEISQDPYQNRIFEMKVMDLFINEYGFSGSHLGGSRKPDGAMYAHGFGVIVDTKAYKDGYNLPISQADEMERYVRENIDRNEHVNSNRWWNIFPEDTNEYKFLFVSGFFKGNFEKQLERISIDTGVQGGALSVEHLLLGAEYIKRGILTLYDFKNSFLNKEIQF

SEQ ID NO: 4 - DNA, 1740 bp, Clostridium botulinum
gtggaatcattaagattatcagacataacaattagaacatttgggtggattcagaatcctagtgattttagtaaattaaaaaaaatagttcagttatttgatcatacatcatctattcatgtggatttgaaagaaaaccgcataccacggttagtggagaaagatgacggacgtgataggtttattgagatattaaatcggattccgttaaagataaagtatattgatttagtaggaacatcatttaaacctagaagtagtggtagatgtaatggaattgctcaagcaatgattgaaggtcaaggtaagagttttactgataattggacagctgatgggtttattaggtgggctcatgcacttggctttatacaatatgattatttagaagatgagttttcaataacacaagcaggctttgatttttcaaggtcaatcaatgatagtgaaggggaaaatgaaatattaatagaggcaatgttgtcttatccacctgcagttagagttttagatttactttctttaggagagcatcttacaaaatttgatattggaaaaaatctgggcttcaatggcgaatcaggatttacatctttacctttaaatatcatgcttcaaacattagcagacaatgatttagtaagtgaaaagactaaaattcgtcaggattgggaaggttcttctgataagtattcacgaatgatagccggctggttatcgaaacttggtttggttaaaaagggaaaaaagtattttgatgtaaatattggaggaataattcatagagaatatatctctcatgcatataaaattactggagaaggtttaaaacaactccgtagggctaaaggaactacaagtgcaaggcgtatagaaaaacgggtttgctgggaaatgttcgccacaaagaatctagataggacatatattcgtacaagaagagcttatattttaaagtttttagaagtttcaagcagcttaattactattgagcaaattaagactaagttattggaaaaaggttatgacgaaacagtagaaactattaaatctgatattaaggggttaattaacattggtttaaatattcaagaaaccactcgaggttattcattaaaggattcaattaatgactttatgattccagtaaccgacttaaatcaaattgttaaaagtagtatagagatgtctaaagctaacatgagagacaatcttcagatgttgcctcatgattatattgagctaattgaaatatcacaagatccatatcaaaatagaatatttgaaatgaaagttatggatttatttattaatgagtatggtttcagtggttcgcacttaggtggaagtaggaaacctgatggtgctatgtatgcacatggttttggtgttattgttgatacaaaagcatataaagatgggtacaatcttcctataagtcaagctgatgaaatggaacgatatgtaagggaaaatattgatagaaatgaacatgtgaactcaaatagatggtggaatatatttcccgaagatacaaatgaatataagtttttattcgtaagtggtttctttaaaggaaattttgagaaacaattagaaaggataagtatagatactggtgtacaaggaggggctttaagtgttgaacatttattattaggtgctgagtacataaagaggggtattcttactttatatgattttaagaatagctttttaaataaggaaattcaattttaa

SEQ ID NO: 5 - protein, 587 aa, Clostridium sp. 7_2_43FAA
MINIIDVNNKTIRTFGWVQNPSNFESLKKVVAIFDNTSKTYNELKDKKIKKLVDERDGQKELLNALNANPLKIKYCNLVGTSFTPRSSARCNGIVQATVKGQRKEFIDDWSSDNFVRWAHALGFIKYNYDTDTFEITDVGRKYVQSEDDSNEESTILEEAMLSYPPVARVLTLLSNGEHLTKYEIGKKLGFVGEAGFTSLPLNVLIMTLATTDEPKEKNKIKTDWDGSSDKYARMISGWLVKLGLLVQRPKLVTVDFGGELYSETIGHAYMITDRGLKAVRRLLGINKVARVSKNVFWEMLATKGIDKNYIRTRRAYILKILIESNKVLTLEDIKGKLKLASINESINTIKDDINGLINTGINIKSETTGYKIYDSINDFIIPKTGDTEGIKSNISLLKDELRGQISHISHEYLSLIDLAFDSKQNRLFEMKVLELLVNEYGFKGRHLGGSRKPDGIVYSTTLEDNFGIIVDTKAYSEGYSLPISQADEMERYVRENSNRDEEVNPNKWWENFSEEVKKYYFVFISGSFKGKFEEQLRRLSMTTGVNGSAVNVVNLLLGAEKIRSGEMTIEELERAMFNNSEFILKY

SEQ ID NO: 6 - DNA, 1764 bp, Clostridium sp. 7_2_43FAA
atgattaacataattgacgtaaataataaaactattagaacttttggatgggttcagaatccaagtaattttgaaagcttaaaaaaagttgtagcaatatttgataatacatcaaagacatataatgaattaaaagataagaaaataaaaaagttagtagacgaaagagatgggcaaaaagaactattaaatgctttaaatgctaatcctttaaagataaagtattgtaatttagtagggacatcttttactccacgaagttctgcaagatgtaatggaatagtacaagccacagtaaaaggacaaagaaaagagttcatagatgattggtcatctgataactttgtaagatgggcacatgctttaggctttattaaatataattatgatacagatacatttgagataaccgatgtaggaagaaagtatgtacagagtgaagatgatagcaatgaggaaagtacaattttagaagaagcaatgttatcatatccaccagtagcaagggttttgacattgctttccaatggagaacatttaacaaaatatgaaataggtaagaaattaggatttgtaggggaagctggttttactagtttgccattgaatgtattaattatgacattagctactacagatgagccgaaggaaaaaaataaaattaaaacagactgggatgggtcttctgataaatatgcaagaatgatttctggttggttagtaaaattaggattattggtacaaagacctaaattggttactgtagattttggtggtgaattatatagcgaaacaataggacatgcttatatgattacggataggggattaaaagctgttagaagattattaggaataaataaagttgcgagggtttcaaaaaatgttttttgggaaatgcttgcaacaaaaggaatagataaaaattatataagaactcgaagagcatatattttaaaaatattaattgaatctaataaggtattaactttagaggatataaaaggaaagttgaaattagcgagtattaatgaatctattaatactattaaagacgatattaatggattaattaatacaggtataaatattaagagtgaaacaactgggtataaaatatatgattcaattaatgattttattatacctaaaacaggagatacagagggaataaagagtaatattagcttattaaaagatgaattaagagggcaaataagtcatatttcacatgagtatttatcattaatagatttagcatttgatagtaagcaaaataggttatttgaaatgaaagttttagagttgttagttaatgagtatggatttaaaggaaggcatctaggtggaagtagaaaacctgatggtatagtttattcaacaactttagaagataattttggaataatagtagatactaaagcttattcagaagggtatagcttacctataagtcaagctgatgaaatggagagatatgttagagaaaactctaatagagatgaggaagtaaaccctaataagtggtgggaaaacttttcagaagaagtcaaaaagtattattttgtattcatatcaggttcctttaagggcaaatttgaagaacaattaagaagattgagcatgactactggggttaacggttcagctgttaatgtagtaaatttattactaggagctgaaaaaataaggtctggagaaatgactattgaagaattagagagagctatgtttaataactcggaatttatattgaagtattaa

SEQ ID NO: 7 - protein, 589 aa, Clostridiales bacterium KA00134
MAERTLGWIQNPSSFENLKNVVSVFDKNTDIYKEILNTKLPKLVKDLDLQNKLISEMKKDPLEMDYVLLKGHGIKSGQKRSDAACSGIVQAAITTQGGRAYTDDWTADGFLRWGISIGLLDYDTENDTVSITKLGEKFVKSNSEDSDKEILISAFLSYPPAVRILTLLESGDHLTKFELGKQLGGLGEAGFTSIPQDLYIQAIELASETDKASIRSNTEGSADKYARMISGWLSKVGLVQRVEKEVSTKIGNVEYMVNIGHSFRITLNGIKELKRARGLSSYPKTDKIVYWQMLATKGKDRDYIRNRRGYIIKAINNRERNLEGIKAYLMENNIDESITTIEDELKVLKAMGLSLKHSRNGYVIDDNIIKLEIPRTKISKTNILELKDKVRDKLKYVDHRYLALIDLAYDGTANRDFEIQTIDLLINELKFKGVRLGESRKPDGIISYNINGVIIDNKAYSTGYNLPINQADEMIRYIEENQTRDEKINSNKWWESFDEKVKDFNYLFVSSFFKGNFKNNLKHIANRTGVNGGAINVENLLYFAEELKAGRISYLDSFKMYNNDEIYLGDISDYSYVKFAAEEEGEYLT

SEQ ID NO: 8 - DNA, 1770 bp, Clostridiales bacterium KA00134
atggcagaaagaacattgggttggatacaaaatccatcaagttttgaaaatttaaaaaatgtagtttctgtttttgataaaaatactgatatatataaggaaatattaaatactaaacttcctaaattagtaaaagatttagatttacaaaataaactcatttcagaaatgaaaaaagatccacttgaaatggactatgttttattaaaaggtcatggtataaaatcaggtcagaaaagatccgatgcagcgtgtagtggtattgttcaagctgccattacaacacaaggcggtagggcttatacagacgattggactgctgatggatttttaagatggggaatatccataggacttttagattatgatacagaaaatgatacagtttctataacaaaactaggagaaaagtttgtaaaatctaattctgaagattcagataaagaaatactaatttcagcctttttgtcatacccaccagccgtaagaattttaactttattggaaagtggagaccatttaacaaaatttgagcttggtaagcaattaggtggacttggagaagctggttttacatcaattcctcaagatttatatattcaagcaatagaacttgcttctgaaacagataaagcaagtattcgatcaaacacagagggatcagctgataaatatgccagaatgatttcaggatggttatctaaggttggtttagttcaaagagttgaaaaagaagtttcaacaaaaattggaaatgttgaatacatggtaaatataggtcattcctttagaattactttgaatggtataaaagaacttaaaagagcaaggggattatcttcatatccaaagactgataaaattgtttattggcaaatgctagcaaccaagggtaaagatagagattatattagaaacagacgtggatatataatcaaagctatcaacaacagagaaagaaatttagaaggcattaaggcttatttaatggaaaataatattgatgaaagtattacaactatagaagacgaactaaaagttcttaaagcaatgggtctttcacttaaacatagtaggaatggctatgtaattgatgataacattataaaattagaaatacctagaactaagatttctaagacaaatatactagaattaaaggataaagtaagagataaattaaaatatgttgaccacagatatcttgcgctaattgatttagcttatgacggaactgccaatagagattttgagattcaaacaatagaccttttaattaatgaacttaagtttaaaggggttcgtctaggagaaagcagaaaaccagatggaattatatcttataatattaatggcgtaattatagataacaaggcttattctacgggttataatctaccaattaatcaagcagatgaaatgattagatatatcgaagaaaatcaaactagagatgaaaaaataaattcaaataaatggtgggaaagctttgatgaaaaagttaaggatttcaactatttatttgtatcatctttctttaagggaaactttaagaataatttgaaacatatagccaatagaactggtgtaaatggtggagctattaatgtagaaaatttattatattttgcagaagaattaaaagctggaagaatatcttatcttgactcatttaaaatgtataacaatgatgaaatatatttaggagatattagtgactatagttatgttaaatttgctgcagaagaagaaggcgaatatttaacataa

SEQ ID NO: 9 - DNA, 38 bp, Artificial
  ND1 substitution forward primer
gatgagatcatcttctaagggcccttcgaaggtaagcc

SEQ ID NO: 10 - DNA, 34 bp, Artificial
  ND1 substitution reverse primer
ctctccctttactaaagctcttgccgcagcaccc

SEQ ID NO: 11 - DNA, 38 bp, Artificial
  ND2 substitution forward primer
aaggagattcagttctaagggcccttcgaaggtaagcc

SEQ ID NO: 12 - DNA, 34 bp, Artificial
  ND2 substitution reverse primer
actacttttaacaatagctcttgccgcagcaccc

SEQ ID NO: 13 - DNA, 38 bp, Artificial
  ND3 substitution forward primer
aacagcgagttcatataagggcccttcgaaggtaagcc

SEQ ID NO: 14 - DNA, 34 bp, Artificial
  ND3 substitution reverse primer
gttactcttgattccagctcttgccgcagcaccc

SEQ ID NO: 15 - DNA, 38 bp, Artificial
  ND4 substitution forward primer
gatgaaatctacctgtaagggcccttcgaaggtaagcc

SEQ ID NO: 16 - DNA, 34 bp, Artificial
  ND4 substitution reverse primer
gtttgtcttggagatagctcttgccgcagcaccc

SEQ ID NO: 17 - DNA, 49 bp, Artificial
  forward primer for linker alteration, ZFN-FokI-GS-F
agaacacacggatccctagtcaaaagtgaactggaggagaagaaatctg

SEQ ID NO: 18 - DNA, 34 bp, Artificial
  reverse primer for linker alteration, ZFN-GS-inverse-R
ggatccgtgtgttctctggtgtctcacgagattg

SEQ ID NO: 19 - DNA, 48 bp, Artificial
  forward primer for linker alteration, ZFN-ND1-GS-F
agaacacacggatccttagtaaagggagagatggagaagaaaaagagc

SEQ ID NO: 20 - DNA, 34 bp, Artificial; identical to SEQ ID NO: 18
  reverse primer for linker alteration, ZFN-GS-inverse-R

SEQ ID NO: 21 - DNA, 47 bp, Artificial
  forward primer for linker alteration, ZFN-ND2-GS-F
agaacacacggatccattgttaaaagtagtattgagatgtccaaggc

SEQ ID NO: 22 - DNA, 34 bp, Artificial; identical to SEQ ID NO: 18
  reverse primer for linker alteration, ZFN-GS-inverse-R

SEQ ID NO: 23 - DNA, 51 bp, Artificial
  forward primer for linker alteration, ZFN-FokI-RPGEKP-F
gacccggggagaagcccctagtcaaaagtgaactggaggagaagaaatctg

SEQ ID NO: 24 - DNA, 44 bp, Artificial
  reverse primer for linker alteration, ZFN-RPGEKP-R
gcttctccccgggtctgtgtgttctctggtgtctcacgagattg

SEQ ID NO: 25 - DNA, 50 bp, Artificial
  forward primer for linker alteration, ZFN-ND1-RPGEKP-F
gacccggggagaagcccttagtaaagggagagatggagaagaaaaagagc

SEQ ID NO: 26 - DNA, 44 bp, Artificial; identical to SEQ ID NO: 24
  reverse primer for linker alteration, ZFN-RPGEKP-R

SEQ ID NO: 27 - DNA, 49 bp, Artificial
  forward primer for linker alteration, ZFN-ND2-RPGEKP-F
gacccggggagaagcccattgttaaaagtagtattgagatgtccaaggc

SEQ ID NO: 28 - DNA, 44 bp, Artificial; identical to SEQ ID NO: 24
  reverse primer for linker alteration, ZFN-RPGEKP-R

SEQ ID NO: 29 - DNA, 55 bp, Artificial
  forward primer for linker alteration, ZFN-FokI-TGPGAAARA-F
cccggggctgcggcaagagctctagtcaaaagtgaactggaggagaagaaatctg

SEQ ID NO: 30 - DNA, 49 bp, Artificial
  reverse primer for linker alteration, ZFN-FokI-TGPGAAARA-R
tgccgcagccccgggacccgtgtgtgttctctggtgtctcacgagattg

SEQ ID NO: 31 - DNA, 54 bp, Artificial
  forward primer for linker alteration, ZFN-ND1-TGPGAAARA-F
cccggggctgcggcaagagctttagtaaagggagagatggagaagaaaaagagc

SEQ ID NO: 32 - DNA, 49 bp, Artificial; identical to SEQ ID NO: 30
  reverse primer for linker alteration, ZFN-FokI-TGPGAAARA-R

SEQ ID NO: 33 - DNA, 53 bp, Artificial
  forward primer for linker alteration, ZFN-ND2-TGPGAAARA-F
cccggggctgcggcaagagctattgttaaaagtagtattgagatgtccaaggc

SEQ ID NO: 34 - DNA, 49 bp, Artificial; identical to SEQ ID NO: 30
  reverse primer for linker alteration, ZFN-FokI-TGPGAAARA-R

SEQ ID NO: 35 - DNA, 59 bp, Artificial
  forward primer for Sharkey mutation introduction in FokI-ND
aaggtaatggaattttttatgaaagtttatggatatagaggtgaacatttgggtggatc

SEQ ID NO: 36 - DNA, 57 bp, Artificial
  reverse primer for Sharkey mutation introduction in FokI-ND
aaattccattaccttcatttcaagaattctatcctgagtaggatttctggcaatttc

SEQ ID NO: 37 - DNA, 59 bp, Artificial
  forward primer for Sharkey mutation introduction in ND1
ttaaggtagtggaatttctgaaagaagtgtacgattacaatggtgagcatctgggcggc

SEQ ID NO: 38 - DNA, 56 bp, Artificial
  reverse primer for Sharkey mutation introduction in ND1
attccactaccttaaactcgaagagtctgttctgcttggggtcctgagcaatttcg

SEQ ID NO: 39 - DNA, 30 bp, Artificial
  forward primer for Sharkey mutation introduction in ND2
tccggggagcatctggggggtagccggaag

SEQ ID NO: 40 - DNA, 34 bp, Artificial
  reverse primer for Sharkey mutation introduction in ND2
cagatgctccccggagaagccatactcgttgatg

SEQ ID NO: 41 - DNA, 19 bp, Artificial
  ZFA substitution forward primer
acgggtgctgcggcaagag

SEQ ID NO: 42 - DNA, 43 bp, Artificial
  ZFA substitution reverse primer
aggtctctcgtggggtctagatttatcgtcgtcatccttgtag

SEQ ID NO: 43 - DNA, 54 bp, Artificial
  forward primer for FokI-DDD mutation introduction
gaagaaaatcaaacacgagacaaacatatcaaccctaatgaatggtggaaagtc

SEQ ID NO: 44 - DNA, 50 bp, Artificial
  reverse primer for FokI-DDD mutation introduction
tgtttgattttcttcgacatagtcttgcatttcatctgcttggccaattg

SEQ ID NO: 45 - DNA, 49 bp, Artificial
  forward primer for ND1-DDD mutation introduction
cgacgaaaataacaatagggacgcaatcatcaaccctaatgagtggtgg

SEQ ID NO: 46 - DNA, 49 bp, Artificial
  reverse primer for ND1-DDD mutation introduction
ttgttattttcgtcgacatagtcttgcatctcatcggcctgagaaattg

SEQ ID NO: 47 - DNA, 49 bp, Artificial
  forward primer for ND2-DDD mutation introduction
tcagggagaacattgacagagacgagcacgtcaattctaaccgctggtg

SEQ ID NO: 48 - DNA, 44 bp, Artificial
  reverse primer for ND2-DDD mutation introduction
caatgttctccctgacgtagtcttccatttcatcggcctggctg

SEQ ID NO: 49 - DNA, 43 bp, Artificial
  forward primer for FokI-RRR vector mutation introduction
ttaaatcggatcactaattgtaatggagctgttcttagtgtag

SEQ ID NO: 50 - DNA, 34 bp, Artificial
  reverse primer for FokI-RRR vector mutation introduction
atttcccgggcttggccaattggcagattataac

SEQ ID NO: 51 - DNA, 38 bp, Artificial
  forward primer for FokI-RRR insert mutation introduction
ccaagcccgggaaatgcaacgatatgtcgaagaaaatc

SEQ ID NO: 52 - DNA, 42 bp, Artificial
  reverse primer for FokI-RRR insert mutation introduction
agtgatccgatttaatcgtgtaagctgagctttgtagtttcc

SEQ ID NO: 53 - DNA, 28 bp, Artificial
  forward primer for ND1-RRR vector mutation introduction
gtgtccagactgaccaagcgcaagggcg

SEQ ID NO: 54 - DNA, 34 bp, Artificial
  reverse primer for ND1-RRR vector mutation introduction
catctcccgggcctgagaaattgggaggctgtag

SEQ ID NO: 55 - DNA, 45 bp, Artificial
  forward primer for ND1-RRR insert mutation introduction
caggcccgggagatgcaaagatatgttgacgaaaataacaatagg

SEQ ID NO: 56 - DNA, 34 bp, Artificial
  reverse primer for ND1-RRR insert mutation introduction
ggtcagtctggacacccttgccagctgtttcttg

SEQ ID NO: 57 - DNA, 28 bp, Artificial
  forward primer for ND2-RRR vector mutation introduction
atctcaagggataccggggtgcagggcg

SEQ ID NO: 58 - DNA, 31 bp, Artificial
  reverse primer for ND2-RRR vector mutation introduction
catttcccgggcctggctgatggggagattg

SEQ ID NO: 59 - DNA, 40 bp, Artificial
  forward primer for ND2-RRR insert mutation introduction
caggcccgggaaatggaaaggtacgtcagggagaacattg

SEQ ID NO: 60 - DNA, 42 bp, Artificial
  reverse primer for ND2-RRR insert mutation introduction
ggtatcccttgagattctttccaactgtttctcaaagtttcc

SEQ ID NO: 61 - DNA, 17 bp, Artificial
  M13-F primer
gtaaaacgacggccagt

SEQ ID NO: 62 - DNA, 24 bp, Cricetulus griseus
accatcttccactctgaagatgga

SEQ ID NO: 63 - DNA, 24 bp, Cricetulus griseus
accatcttcaagagagaagatggc

SEQ ID NO: 64 - DNA, 24 bp, Cricetulus griseus
accatcttccttgatgaagatgcc

SEQ ID NO: 65 - DNA, 24 bp, Cricetulus griseus
gtcaccttcaagtctgaagatggt

SEQ ID NO: 66 - DNA, 24 bp, Cricetulus griseus
ttcaccttcttaagtgaagatggt

SEQ ID NO: 67 - protein, 195 aa, Artificial
  FokI-DDD amino acid sequence
LVKSELEEKKSELRHKLKYVPHEYIELIEIARNSTQDRILEMKVMEFFMKVYGYRGKHLGGSRKPDGAIYTVGSPIDYGVIVDTKAYSGGYNLPIGQADEMQDYVEENQTRDKHINPNEWWKVYPSSVTEFKFLFVSGHFKGNYKAQLTRLNHITNCNGAVLSVEELLIGGEMIKAGTLTLEEVRRKFNNGEINF

SEQ ID NO: 68 - protein, 195 aa, Artificial
  FokI-RRR amino acid sequence
LVKSELEEKKSELRHKLKYVPHEYIELIEIARNSTQDRILEMKVMEFFMKVYGYRGKHLGGSRKPDGAIYTVGSPIDYGVIVDTKAYSGGYNLPIGQAREMQRYVEENQTRNKHINPNEWWKVYPSSVTEFKFLFVSGHFKGNYKAQLTRLNRITNCNGAVLSVEELLIGGEMIKAGTLTLEEVRRKFNNGEINF

SEQ ID NO: 69 - protein, 195 aa, Artificial
  ND1-DDD amino acid sequence
LVKGEMEKKKSDLRHKLKHVPHEYIELIEIAQDSKQNRLFEFKVVEFLKEVYDYNGKHLGGSRKPDGALYTNGLKTDYGIILDTKAYKDGYSLPISQADEMQDYVDENNNRDAIINPNEWWKVYPNSILDFKFLFVSGFFKGDYKKQLARVSNLTKRKGAVLSVEQLLLGGEKIKDGSLTLEDVGDKFNNDEIIF

SEQ ID NO: 70 - protein, 195 aa, Artificial
  ND1-RRR amino acid sequence
LVKGEMEKKKSDLRHKLKHVPHEYIELIEIAQDSKQNRLFEFKVVEFLKEVYDYNGKHLGGSRKPDGALYTNGLKTDYGIILDTKAYKDGYSLPISQAREMQRYVDENNNRNAIINPNEWWKVYPNSILDFKFLFVSGFFKGDYKKQLARVSRLTKRKGAVLSVEQLLLGGEKIKDGSLTLEDVGDKFNNDEIIF

SEQ ID NO: 71 - protein, 191 aa, Artificial
  ND2-DDD amino acid sequence
IVKSSIEMSKANMRDNLQMLPHDYIELIEISQDPYQNRIFEMKVMDLFINEYGFSGSHLGGSRKPDGAMYAHGFGVIVDTKAYKDGYNLPISQADEMEDYVRENIDRDEHVNSNRWWNIFPEDTNEYKFLFVSGFFKGNFEKQLERISIDTGVQGGALSVEHLLLGAEYIKRGILTLYDFKNSFLNKEIQF

SEQ ID NO: 72 - protein, 191 aa, Artificial
  ND2-RRR amino acid sequence
IVKSSIEMSKANMRDNLQMLPHDYIELIEISQDPYQNRIFEMKVMDLFINEYGFSGSHLGGSRKPDGAMYAHGFGVIVDTKAYKDGYNLPISQAREMERYVRENIDRNEHVNSNRWWNIFPEDTNEYKFLFVSGFFKGNFEKQLERISRDTGVQGGALSVEHLLLGAEYIKRGILTLYDFKNSFLNKEIQF

SEQ ID NO: 73 - protein, 195 aa, Artificial
  FokI-S418P/K441E amino acid sequence
LVKSELEEKKSELRHKLKYVPHEYIELIEIARNPTQDRILEMKVMEFFMKVYGYRGEHLGGSRKPDGAIYTVGSPIDYGVIVDTKAYSGGYNLPIGQADEMQRYVEENQTRNKHINPNEWWKVYPSSVTEFKFLFVSGHFKGNYKAQLTRLNHITNCNGAVLSVEELLIGGEMIKAGTLTLEEVRRKFNNGEINF

SEQ ID NO: 74 - protein, 195 aa, Artificial
  ND1-S418P/K441E amino acid sequence
LVKGEMEKKKSDLRHKLKHVPHEYIELIEIAQDPKQNRLFEFKVVEFLKEVYDYNGEHLGGSRKPDGALYTNGLKTDYGIILDTKAYKDGYSLPISQADEMQRYVDENNNRNAIINPNEWWKVYPNSILDFKFLFVSGFFKGDYKKQLARVSNLTKRKGAVLSVEQLLLGGEKIKDGSLTLEDVGDKFNNDEIIF

SEQ ID NO: 75 - protein, 191 aa, Artificial
  ND2-S441E amino acid sequence
IVKSSIEMSKANMRDNLQMLPHDYIELIEISQDPYQNRIFEMKVMDLFINEYGFSGEHLGGSRKPDGAMYAHGFGVIVDTKAYKDGYNLPISQADEMERYVRENIDRNEHVNSNRWWNIFPEDTNEYKFLFVSGFFKGNFEKQLERISIDTGVQGGALSVEHLLLGAEYIKRGILTLYDFKNSFLNKEIQF

SEQ ID NO: 76 - DNA, 34 bp, Artificial
  FokI-cleaved CHO-K1 ZFA36-ZFA36 target 1st site
cagccaccatcttccactctgaagatggacaggt

SEQ ID NO: 77 - DNA, 35 bp, Artificial
  FokI-cleaved CHO-K1 ZFA36-ZFA36 target 1st site
cagccaccatcttccactcttgaagatggacaggt

SEQ ID NO: 78 - DNA, 38 bp, Artificial
  FokI-cleaved CHO-K1 ZFA36-ZFA36 target 1st site
cagccaccatcttccactcactctgaagatggacaggt

SEQ ID NO: 79 - DNA, 34 bp, Artificial; identical to SEQ ID NO: 76
  ND1-cleaved CHO-K1 ZFA36-ZFA36 target 1st site

SEQ ID NO: 80 - DNA, 35 bp, Artificial
  ND1-cleaved CHO-K1 ZFA36-ZFA36 target 1st site
cagccaccatcttccaactctgaagatggacaggt

SEQ ID NO: 81 - DNA, 36 bp, Artificial
  ND1-cleaved CHO-K1 ZFA36-ZFA36 target 1st site
cagccaccatcttccactctctgaagatggacaggt

SEQ ID NO: 82 - DNA, 38 bp, Artificial; identical to SEQ ID NO: 78
  ND1-cleaved CHO-K1 ZFA36-ZFA36 target 1st site

SEQ ID NO: 83 - DNA, 32 bp, Artificial
  ND1-cleaved CHO-K1 ZFA36-ZFA36 target 1st site
cagccaccatcttcctctgaagatggacaggt

SEQ ID NO: 84 - DNA, 25 bp, Artificial
  ND1-cleaved CHO-K1 ZFA36-ZFA36 target 1st site
cagcccactctgaagatggacaggt

SEQ ID NO: 85 - DNA, 34 bp, Artificial; identical to SEQ ID NO: 76
  ND2-cleaved CHO-K1 ZFA36-ZFA36 target 1st site

SEQ ID NO: 86 - DNA, 35 bp, Artificial; identical to SEQ ID NO: 77
  ND2-cleaved CHO-K1 ZFA36-ZFA36 target 1st site

SEQ ID NO: 87 - DNA, 36 bp, Artificial; identical to SEQ ID NO: 81
  ND2-cleaved CHO-K1 ZFA36-ZFA36 target 1st site

SEQ ID NO: 88 - DNA, 32 bp, Artificial; identical to SEQ ID NO: 83
  ND2-cleaved CHO-K1 ZFA36-ZFA36 target 1st site

SEQ ID NO: 89 - DNA, 30 bp, Artificial
  ND2-cleaved CHO-K1 ZFA36-ZFA36 target 1st site
cagccaccatctttctgaagatggacaggt

SEQ ID NO: 90 - DNA, 34 bp, Artificial; identical to SEQ ID NO: 76
  ND3-cleaved CHO-K1 ZFA36-ZFA36 target 1st site

SEQ ID NO: 91 - DNA, 34 bp, Artificial; identical to SEQ ID NO: 76
  ND4-cleaved CHO-K1 ZFA36-ZFA36 target 1st site

SEQ ID NO: 92 - DNA, 34 bp, Artificial
  FokI-cleaved CHO-K1 ZFA36-ZFA36 target 2nd site
accttaccatcttcaagagagaagatggcttaaa

SEQ ID NO: 93 - DNA, 36 bp, Artificial
  FokI-cleaved CHO-K1 ZFA36-ZFA36 target 2nd site
accttaccatcttcaagagagagaagatggcttaaa

SEQ ID NO: 94 - DNA, 38 bp, Artificial
  FokI-cleaved CHO-K1 ZFA36-ZFA36 target 2nd site
accttaccatcttcaagagagagagaagatggcttaaa

SEQ ID NO: 95 - DNA, 39 bp, Artificial
  FokI-cleaved CHO-K1 ZFA36-ZFA36 target 2nd site
accttaccatcttcaagaggagagagaagatggcttaaa

SEQ ID NO: 96 - DNA, 32 bp, Artificial
  FokI-cleaved CHO-K1 ZFA36-ZFA36 target 2nd site
accttaccatcttcaagagaagatggcttaaa

SEQ ID NO: 97 - DNA, 268 bp, Artificial
  FokI-cleaved CHO-K1 ZFA36-ZFA36 target 2nd site
accttaccatcttcaagagcatgaacacatcaccattcattaccaaaaataaaaaatcttactatgaagagctcttgggaatgggagtgttagcctaatgagagaacagacacttagcatattctaggccttaggatcagtcaccaccaccaaaaaacaaacaaacaaaaaacttaacacatgttcatccccagttagtttaagtcagggaccaagtaagattcccattttgcagtagaatggtatcacttaggtaagatggcttaaa

SEQ ID NO: 98 - DNA, 34 bp, Artificial; identical to SEQ ID NO: 92
  ND1-cleaved CHO-K1 ZFA36-ZFA36 target 2nd site

SEQ ID NO: 99 - DNA, 36 bp, Artificial; identical to SEQ ID NO: 93
  ND1-cleaved CHO-K1 ZFA36-ZFA36 target 2nd site

SEQ ID NO: 100 - DNA, 38 bp, Artificial; identical to SEQ ID NO: 94
  ND1-cleaved CHO-K1 ZFA36-ZFA36 target 2nd site

SEQ ID NO: 101 - DNA, 32 bp, Artificial
  ND1-cleaved CHO-K1 ZFA36-ZFA36 target 2nd site
accttaccatcttcaatagaagatggcttaaa

SEQ ID NO: 102 - DNA, 30 bp, Artificial
  ND1-cleaved CHO-K1 ZFA36-ZFA36 target 2nd site
accttaccatcttcaagaggatggcttaaa

SEQ ID NO: 103 - DNA, 34 bp, Artificial; identical to SEQ ID NO: 92
  ND2-cleaved CHO-K1 ZFA36-ZFA36 target 2nd site

SEQ ID NO: 104 - DNA, 35 bp, Artificial
  ND2-cleaved CHO-K1 ZFA36-ZFA36 target 2nd site
accttaccatcttcaaagagagaagatggcttaaa

SEQ ID NO: 105 - DNA, 36 bp, Artificial; identical to SEQ ID NO: 93
  ND2-cleaved CHO-K1 ZFA36-ZFA36 target 2nd site

SEQ ID NO: 106 - DNA, 38 bp, Artificial; identical to SEQ ID NO: 94
  ND2-cleaved CHO-K1 ZFA36-ZFA36 target 2nd site

SEQ ID NO: 107 - DNA, 105 bp, Artificial
  ND2-cleaved CHO-K1 ZFA36-ZFA36 target 2nd site
accttaccatcttcaggtcttcctggtgtagaatccctagtctttggtggtgtcatataagtcttttgttgttgaatgcattcttaagagagaagatggcttaaa

SEQ ID NO: 108 - DNA, 34 bp, Artificial; identical to SEQ ID NO: 92
  ND3-cleaved CHO-K1 ZFA36-ZFA36 target 2nd site

SEQ ID NO: 109 - DNA, 36 bp, Artificial; identical to SEQ ID NO: 93
  ND3-cleaved CHO-K1 ZFA36-ZFA36 target 2nd site

SEQ ID NO: 110 - DNA, 32 bp, Artificial; identical to SEQ ID NO: 96
  ND3-cleaved CHO-K1 ZFA36-ZFA36 target 2nd site

SEQ ID NO: 111 - DNA, 26 bp, Artificial
  ND3-cleaved CHO-K1 ZFA36-ZFA36 target 2nd site
accttaccatcttcagttggcttaaa

SEQ ID NO: 112 - DNA, 34 bp, Artificial
  ND4-cleaved CHO-K1 ZFA36-ZFA36 target 2nd site
cagccaccatcttcaagagagaagatggcttaaa

SEQ ID NO: 113 - DNA, 30 bp, Artificial
  forward primer for vector amplification for ptTALE-ND substitution, ptTALEN-inverse-F
taaaaaatcagcctcgactgtgccttctag

SEQ ID NO: 114 - DNA, 22 bp, Artificial
  reverse primer for vector amplification for ptTALE-ND substitution, NC-inverse-R_2
ctgggatctgatcaattccggc

SEQ ID NO: 115 - DNA, 48 bp, Artificial
  forward primer for insert amplification for ptTALE-ND substitution, ND1-NC-F_v2
ttgatcagatcccagttagtaaagggagagatggagaagaaaaagagc

SEQ ID NO: 116 - DNA, 46 bp, Artificial
  reverse primer for insert amplification for ptTALE-ND substitution, ND1-ptTALEN-R
gaggctgattttttagaagatgatctcatcgttgttgaacttatcc

SEQ ID NO: 117 - DNA, 50 bp, Cricetulus griseus
tgcccagaagactcccgcccatctcccagaaagcctcgacttgcagatca

SEQ ID NO: 118 - DNA, 51 bp, Cricetulus griseus
tgaaccaggctatgacctagatttattttgtattcctaatcactatgtcga

SEQ ID NO: 119 - protein, 318 aa, Artificial Sequence
  ZF(ZFA36A)-ND1 amino acid sequence
MGHHHHHHMRLEPKKKRKVAAADYKDDDDKSRPGEKPYKCPECGKSFSTSGHLVRHQRTHTGEKPYKCPECGKSFSTSGNLVRHQRTHTGEKPYKCPECGKSFSQSSNLVRHQRTHTGAAARALVKGEMEKKKSDLRHKLKHVPHEYIELIEIAQDSKQNRLFEFKVVEFLKEVYDYNGKHLGGSRKPDGALYTNGLKTDYGIILDTKAYKDGYSLPISQADEMQRYVDENNNRNAIINPNEWWKVYPNSILDFKFLFVSGFFKGDYKKQLARVSNLTKRKGAVLSVEQLLLGGEKIKDGSLTLEDVGDKFNNDEIIF

SEQ ID NO: 120 - protein, 318 aa, Artificial Sequence
  ZF(ZFL1)-ND1 amino acid sequence
MGHHHHHHMRLEPKKKRKVAAADYKDDDDKSRPHERPFQCRICMRNFSDRSNLTRHTRTHTGEKPFQCRICMRNFSLRHHLTRHLRTHTGEKPFQCRICMRNFSQKANLTRHLRTHTGAAARALVKGEMEKKKSDLRHKLKHVPHEYIELIEIAQDSKQNRLFEFKVVEFLKEVYDYNGKHLGGSRKPDGALYTNGLKTDYGIILDTKAYKDGYSLPISQADEMQRYVDENNNRNAIINPNEWWKVYPNSILDFKFLFVSGFFKGDYKKQLARVSNLTKRKGAVLSVEQLLLGGEKIKDGSLTLEDVGDKFNNDEIIF

SEQ ID NO: 121 - protein, 318 aa, Artificial Sequence
  ZF(ZFA36A)-FokI amino acid sequence
MGHHHHHHMRLEPKKKRKVAAADYKDDDDKSRPGEKPYKCPECGKSFSTSGHLVRHQRTHTGEKPYKCPECGKSFSTSGNLVRHQRTHTGEKPYKCPECGKSFSQSSNLVRHQRTHTGAAARALVKSELEEKKSELRHKLKYVPHEYIELIEIARNSTQDRILEMKVMEFFMKVYGYRGKHLGGSRKPDGAIYTVGSPIDYGVIVDTKAYSGGYNLPIGQADEMQRYVEENQTRNKHINPNEWWKVYPSSVTEFKFLFVSGHFKGNYKAQLTRLNHITNCNGAVLSVEELLIGGEMIKAGTLTLEEVRRKFNNGEINF

SEQ ID NO: 122 - protein, 318 aa, Artificial Sequence
  ZF(ZFL1)-FokI amino acid sequence
MGHHHHHHMRLEPKKKRKVAAADYKDDDDKSRPHERPFQCRICMRNFSDRSNLTRHTRTHTGEKPFQCRICMRNFSLRHHLTRHLRTHTGEKPFQCRICMRNFSQKANLTRHLRTHTGAAARALVKSELEEKKSELRHKLKYVPHEYIELIEIARNSTQDRILEMKVMEFFMKVYGYRGKHLGGSRKPDGAIYTVGSPIDYGVIVDTKAYSGGYNLPIGQADEMQRYVEENQTRNKHINPNEWWKVYPSSVTEFKFLFVSGHFKGNYKAQLTRLNHITNCNGAVLSVEELLIGGEMIKAGTLTLEEVRRKFNNGEINF